European Patent Application EP 4 711 744 A1, published March 18, 2026. Title: SYSTEME D'AUTHENTIFICATION PAR ANALYSE DES SPECTRES DE DICHROISME CIRCULAIRE DE MOLECULES BIOLOGIQUES OU ORGANIQUES. Applicant: CENTRE NATIONAL DE LA RECHERCHE SCIENTIFIQUE. The sequence listing filed with the application follows.

SEQUENCE LISTING (1 sequence)

SEQ ID NO: 1 - protein, 21 aa, Synthetic construct
TPEEIARWREERRKNYPTLAN